European Patent Application EP 4 461 747 A1, published November 13, 2024. Title: 靶向MSLN的抗原结合蛋白及其应用. Applicant: 原启生物科技（上海）有限责任公司. The sequence listing filed with the application follows.

SEQUENCE LISTING (70 sequences)

SEQ ID NO: 1 - protein, 10 aa, synthetic construct
  REGION 1..10: note = MSLN16 HCDR3
TINSASDYDY

SEQ ID NO: 2 - protein, 17 aa, synthetic construct
  REGION 1..17: note = MSLN16 HCDR2
YISWGGSRTYYPDSVEG

SEQ ID NO: 3 - protein, 5 aa, synthetic construct
  REGION 1..5: note = MSLN16 HCDR1
NYNMG

SEQ ID NO: 4 - protein, 30 aa, synthetic construct
  REGION 1..30: note = MSLN16H-FR1
EVQLVESGGGLVQPGGSLRLSCAASGRILS

SEQ ID NO: 5 - protein, 14 aa, synthetic construct
  REGION 1..14: note = MSLN16, MSLN3, MSLN10, MSLN27, MSLN36, MSLN41, MSLN42 H-FR2
WFRQAPGKGRELVA

SEQ ID NO: 6 - protein, 32 aa, synthetic construct
  REGION 1..32: note = MSLN16, MSLN3, MSLN10, MSLN27, MSLN36, MSLN41, MSLN42 H-FR3
RFTISRDNAKRMVYLQMNSLRAEDTAVYYCAA

SEQ ID NO: 7 - protein, 11 aa, synthetic construct
  REGION 1..11: note = MSLN16, MSLN3, MSLN10, MSLN27, MSLN36, MSLN41, MSLN42 H-FR4
WGQGTQVTVSS

SEQ ID NO: 8 - protein, 119 aa, synthetic construct
  REGION 1..119: note = MSLN16 VHH
EVQLVESGGGLVQPGGSLRLSCAASGRILSNYNMGWFRQAPGKGRELVAYISWGGSRTYYPDSVEGRFTISRDNAKRMVYLQMNSLRAEDTAVYYCAATINSASDYDYWGQGTQVTVSS

SEQ ID NO: 9 - protein, 12 aa, synthetic construct
  REGION 1..12: note = MSLN3 HCDR3
SIKTADPDDYDY

SEQ ID NO: 10 - protein, 17 aa, synthetic construct
  REGION 1..17: note = MSLN3 HCDR2
YISWRGGSTYYPDSVEG

SEQ ID NO: 11 - protein, 5 aa, synthetic construct
  REGION 1..5: note = MSLN3 HCDR1
RYNMG

SEQ ID NO: 12 - protein, 30 aa, synthetic construct
  REGION 1..30: note = MSLN3 H-FR1
EVQLVESGGGLVQPGGSLRLSCAASGNTLS

SEQ ID NO: 13 - protein, 121 aa, synthetic construct
  REGION 1..121: note = MSLN3 VHH
EVQLVESGGGLVQPGGSLRLSCAASGNTLSRYNMGWFRQAPGKGRELVAYISWRGGSTYYPDSVEGRFTISRDNAKRMVYLQMNSLRAEDTAVYYCAASIKTADPDDYDYWGQGTQVTVSS

SEQ ID NO: 14 - protein, 15 aa, synthetic construct
  REGION 1..15: note = MSLN10 HCDR3
RRIGPVYDPYSVYNY

SEQ ID NO: 15 - protein, 17 aa, synthetic construct
  REGION 1..17: note = MSLN10 HCDR2
GITSSGSGTYYPDSVEG

SEQ ID NO: 16 - protein, 5 aa, synthetic construct
  REGION 1..5: note = MSLN10 HCDR1
TYAMG

SEQ ID NO: 17 - protein, 30 aa, synthetic construct
  REGION 1..30: note = MSLN10 H-FR1
EVQLVESGGGLVQPGGSLRLSCAASGDTLS

SEQ ID NO: 18 - protein, 124 aa, synthetic construct
  REGION 1..124: note = MSLN10 VHH
EVQLVESGGGLVQPGGSLRLSCAASGDTLSTYAMGWFRQAPGKGRELVAGITSSGSGTYYPDSVEGRFTISRDNAKRMVYLQMNSLRAEDTAVYYCAARRIGPVYDPYSVYNYWGQGTQVTVSS

SEQ ID NO: 19 - protein, 15 aa, synthetic construct
  REGION 1..15: note = MSLN27 HCDR3
GTARIDYLSQDGYNY

SEQ ID NO: 20 - protein, 17 aa, synthetic construct
  REGION 1..17: note = MSLN27 HCDR2
AISWRGGYTYYPDSVEG

SEQ ID NO: 21 - protein, 5 aa, synthetic construct
  REGION 1..5: note = MSLN27 HCDR1
TNAMG

SEQ ID NO: 22 - protein, 30 aa, synthetic construct
  REGION 1..30: note = MSLN27 H-FR1
EVQLVESGGGLVQPGGSLRLSCAASGLIFS

SEQ ID NO: 23 - protein, 124 aa, synthetic construct
  REGION 1..124: note = MSLN27 VHH
EVQLVESGGGLVQPGGSLRLSCAASGLIFSTNAMGWFRQAPGKGRELVAAISWRGGYTYYPDSVEGRFTISRDNAKRMVYLQMNSLRAEDTAVYYCAAGTARIDYLSQDGYNYWGQGTQVTVSS

SEQ ID NO: 24 - protein, 19 aa, synthetic construct
  REGION 1..19: note = MSLN36 HCDR3
KRAYWGSDGDYQGYYYYDY

SEQ ID NO: 25 - protein, 17 aa, synthetic construct
  REGION 1..17: note = MSLN36 HCDR2
AITASGGNTYYPDSVEG

SEQ ID NO: 26 - protein, 5 aa, synthetic construct
  REGION 1..5: note = MSLN36 HCDR1
NYVMG

SEQ ID NO: 27 - protein, 30 aa, synthetic construct
  REGION 1..30: note = MSLN36 H-FR1
EVQLVESGGGLVQPGGSLRLSCAASGITFS

SEQ ID NO: 28 - protein, 128 aa, synthetic construct
  REGION 1..128: note = MSLN36 VHH
EVQLVESGGGLVQPGGSLRLSCAASGITFSNYVMGWFRQAPGKGRELVAAITASGGNTYYPDSVEGRFTISRDNAKRMVYLQMNSLRAEDTAVYYCAAKRAYWGSDGDYQGYYYYDYWGQGTQVTVSS

SEQ ID NO: 29 - protein, 19 aa, synthetic construct
  REGION 1..19: note = MSLN41 HCDR3
ATARVYADDSYLNESGYDY

SEQ ID NO: 30 - protein, 17 aa, synthetic construct
  REGION 1..17: note = MSLN41 HCDR2
AITWRGGYTYYPDSVEG

SEQ ID NO: 31 - protein, 5 aa, synthetic construct
  REGION 1..5: note = MSLN41 HCDR1
YNAMG

SEQ ID NO: 32 - protein, 30 aa, synthetic construct
  REGION 1..30: note = MSLN41 H-FR1
EVQLVESGGGLVQPGGSLRLSCAASGRTFS

SEQ ID NO: 33 - protein, 128 aa, synthetic construct
  REGION 1..128: note = MSLN41 VHH
EVQLVESGGGLVQPGGSLRLSCAASGRTFSYNAMGWFRQAPGKGRELVAAITWRGGYTYYPDSVEGRFTISRDNAKRMVYLQMNSLRAEDTAVYYCAAATARVYADDSYLNESGYDYWGQGTQVTVSS

SEQ ID NO: 34 - protein, 19 aa, synthetic construct
  REGION 1..19: note = MSLN42 HCDR3
RFAPDPAFSVYWSENYYDY

SEQ ID NO: 35 - protein, 17 aa, synthetic construct
  REGION 1..17: note = MSLN42 HCDR2
AITPRGSGTYYPDSVEG

SEQ ID NO: 36 - protein, 5 aa, synthetic construct
  REGION 1..5: note = MSLN42 HCDR1
SNVMG

SEQ ID NO: 37 - protein, 30 aa, synthetic construct
  REGION 1..30: note = MSLN42 H-FR1
EVQLVESGGGLVQPGGSLRLSCAASGRTLS

SEQ ID NO: 38 - protein, 128 aa, synthetic construct
  REGION 1..128: note = MSLN42 VHH
EVQLVESGGGLVQPGGSLRLSCAASGRTLSSNVMGWFRQAPGKGRELVAAITPRGSGTYYPDSVEGRFTISRDNAKRMVYLQMNSLRAEDTAVYYCAARFAPDPAFSVYWSENYYDYWGQGTQVTVSS

SEQ ID NO: 39 - protein, 42 aa, synthetic construct
  REGION 1..42: note = 4-1BB co-stimulatory domain
KRGRKKLLYIFKQPFMRPVQTTQEEDGCSCRFPEEEEGGCEL

SEQ ID NO: 40 - protein, 24 aa, synthetic construct
  REGION 1..24: note = CD8 transmembrane domain
IYIWAPLAGTCGVLLLSLVITLYC

SEQ ID NO: 41 - protein, 112 aa, synthetic construct
  REGION 1..112: note = CD3zeta intracellular signaling domain
RVKFSRSADAPAYQQGQNQLYNELNLGRREEYDVLDKRRGRDPEMGGKPRRKNPQEGLYNELQKDKMAEAYSEIGMKGERRRGKGHDGLYQGLSTATKDTYDALHMQALPPR

SEQ ID NO: 42 - protein, 45 aa, synthetic construct
  REGION 1..45: note = CD8 hinge region
TTTPAPRPPTPAPTIASQPLSLRPEACRPAAGGAVHTRGLDFACD

SEQ ID NO: 43 - protein, 21 aa, synthetic construct
  REGION 1..21: note = CD8 signal peptide
MALPVTALLLPLALLLHAARP

SEQ ID NO: 44 - protein, 398 aa, synthetic construct
  REGION 1..398: note = Ori amino acid sequence
MGAVLRSLLACSFCVLLRAEQKLISEEDLEPPTCSPQQFTCFTGEIDCIPVAWRCDGFTECEDHSDELNCPVCSESQFQCASGQCIDGALRCNGDANCQDKSDEKNCEVLCLIDQFRCANGQCIGKHKKCDHNVDCSDKSDELDCYPTEEPAPQATNTVGSVIGVIVTIFVSGTVYFICQRMLCPRMKGDGETMTNDYVVHGPASVPLGYVPHPSSLSGSLPGMSRGKSMISSLSIMGGSSGPPYDRAHVTGASSSSSSSTKGTYFPAILNPPPSPATERSHYTMEFGYSSNSPSTHRSYSYRPYSYRHFAPPTTPCSTDVCDSDYAPSRRMTSVATAKGYTSDLNYDSEPVPPPPTPRSQYLSAEENYESCPPSPYTERSYSHHLYPPPPSPCTDSS

SEQ ID NO: 45 - DNA, 1194 bp, synthetic construct
  misc_feature 1..1194: note = Ori nucleotide sequence
  source 1..1194: mol_type = other DNA
atgggggccgtcctgaggagcctcctggcctgcagcttctgtgtgctcctgagagcggagcagaaactcatctctgaagaggatctggaacctccaacatgttctcctcagcagtttacttgtttcacgggggaaattgactgtatccctgtggcttggcggtgcgatgggtttactgaatgtgaagaccacagtgatgaactcaattgtcctgtatgctcagagtcccagttccagtgtgccagtgggcagtgtattgatggtgccctccgatgcaatggagatgcaaactgccaggacaaatcagatgagaagaactgtgaagtgctttgtttaattgatcagttccgctgtgccaatggtcagtgcattggaaagcacaagaagtgtgatcataatgtggattgcagtgacaagtcagatgaactggattgttatccgactgaagaaccagcaccacaggccaccaatacagttggttctgttattggcgtaattgtcaccatttttgtgtctggaactgtatactttatctgccagaggatgttgtgtccacgtatgaagggagatggggaaactatgactaatgactatgtagttcatggaccagcttctgtgcctcttggttatgtgccacacccaagttctttgtcaggatctcttccaggaatgtctcgaggtaaatcaatgatcagctccctcagtatcatggggggaagcagtggacccccctatgaccgagcccatgttacaggagcatcatcaagtagttcttcaagcaccaaaggcacttacttccctgcaattttgaaccctccaccatccccagccacagagcgatcacattacactatggaatttggatattcttcaaacagtccttccactcataggtcatacagctacaggccatatagctaccggcactttgcaccccccaccacaccctgcagcacagatgtttgtgacagtgactatgctcctagtcggagaatgacctcagtggcaacagccaagggctataccagtgacttgaactatgattcagaacctgtgcccccacctcccacaccccgaagccaatacttgtcagcagaggagaactatgaaagctgcccaccttctccatacacagagaggagctattctcatcacctctacccaccgccaccctctccctgtacagactcctcc

SEQ ID NO: 46 - protein, 18 aa, synthetic construct
  REGION 1..18: note = cleavage peptide
EGRGSLLTCGDVEENPGP

SEQ ID NO: 47 - protein, 758 aa, synthetic construct
  REGION 1..758: note = MSLN16 CAR
EVQLVESGGGLVQPGGSLRLSCAASGRILSNYNMGWFRQAPGKGRELVAYISWGGSRTYYPDSVEGRFTISRDNAKRMVYLQMNSLRAEDTAVYYCAATINSASDYDYWGQGTQVTVSSTTTPAPRPPTPAPTIASQPLSLRPEACRPAAGGAVHTRGLDFACDIYIWAPLAGTCGVLLLSLVITLYCKRGRKKLLYIFKQPFMRPVQTTQEEDGCSCRFPEEEEGGCELRVKFSRSADAPAYQQGQNQLYNELNLGRREEYDVLDKRRGRDPEMGGKPRRKNPQEGLYNELQKDKMAEAYSEIGMKGERRRGKGHDGLYQGLSTATKDTYDALHMQALPPREGRGSLLTCGDVEENPGPMGAVLRSLLACSFCVLLRAEQKLISEEDLEPPTCSPQQFTCFTGEIDCIPVAWRCDGFTECEDHSDELNCPVCSESQFQCASGQCIDGALRCNGDANCQDKSDEKNCEVLCLIDQFRCANGQCIGKHKKCDHNVDCSDKSDELDCYPTEEPAPQATNTVGSVIGVIVTIFVSGTVYFICQRMLCPRMKGDGETMTNDYVVHGPASVPLGYVPHPSSLSGSLPGMSRGKSMISSLSIMGGSSGPPYDRAHVTGASSSSSSSTKGTYFPAILNPPPSPATERSHYTMEFGYSSNSPSTHRSYSYRPYSYRHFAPPTTPCSTDVCDSDYAPSRRMTSVATAKGYTSDLNYDSEPVPPPPTPRSQYLSAEENYESCPPSPYTERSYSHHLYPPPPSPCTDSS

SEQ ID NO: 48 - protein, 760 aa, synthetic construct
  REGION 1..760: note = MSLN3 CAR
EVQLVESGGGLVQPGGSLRLSCAASGNTLSRYNMGWFRQAPGKGRELVAYISWRGGSTYYPDSVEGRFTISRDNAKRMVYLQMNSLRAEDTAVYYCAASIKTADPDDYDYWGQGTQVTVSSTTTPAPRPPTPAPTIASQPLSLRPEACRPAAGGAVHTRGLDFACDIYIWAPLAGTCGVLLLSLVITLYCKRGRKKLLYIFKQPFMRPVQTTQEEDGCSCRFPEEEEGGCELRVKFSRSADAPAYQQGQNQLYNELNLGRREEYDVLDKRRGRDPEMGGKPRRKNPQEGLYNELQKDKMAEAYSEIGMKGERRRGKGHDGLYQGLSTATKDTYDALHMQALPPREGRGSLLTCGDVEENPGPMGAVLRSLLACSFCVLLRAEQKLISEEDLEPPTCSPQQFTCFTGEIDCIPVAWRCDGFTECEDHSDELNCPVCSESQFQCASGQCIDGALRCNGDANCQDKSDEKNCEVLCLIDQFRCANGQCIGKHKKCDHNVDCSDKSDELDCYPTEEPAPQATNTVGSVIGVIVTIFVSGTVYFICQRMLCPRMKGDGETMTNDYVVHGPASVPLGYVPHPSSLSGSLPGMSRGKSMISSLSIMGGSSGPPYDRAHVTGASSSSSSSTKGTYFPAILNPPPSPATERSHYTMEFGYSSNSPSTHRSYSYRPYSYRHFAPPTTPCSTDVCDSDYAPSRRMTSVATAKGYTSDLNYDSEPVPPPPTPRSQYLSAEENYESCPPSPYTERSYSHHLYPPPPSPCTDSS

SEQ ID NO: 49 - protein, 763 aa, synthetic construct
  REGION 1..763: note = MSLN10 CAR
EVQLVESGGGLVQPGGSLRLSCAASGDTLSTYAMGWFRQAPGKGRELVAGITSSGSGTYYPDSVEGRFTISRDNAKRMVYLQMNSLRAEDTAVYYCAARRIGPVYDPYSVYNYWGQGTQVTVSSTTTPAPRPPTPAPTIASQPLSLRPEACRPAAGGAVHTRGLDFACDIYIWAPLAGTCGVLLLSLVITLYCKRGRKKLLYIFKQPFMRPVQTTQEEDGCSCRFPEEEEGGCELRVKFSRSADAPAYQQGQNQLYNELNLGRREEYDVLDKRRGRDPEMGGKPRRKNPQEGLYNELQKDKMAEAYSEIGMKGERRRGKGHDGLYQGLSTATKDTYDALHMQALPPREGRGSLLTCGDVEENPGPMGAVLRSLLACSFCVLLRAEQKLISEEDLEPPTCSPQQFTCFTGEIDCIPVAWRCDGFTECEDHSDELNCPVCSESQFQCASGQCIDGALRCNGDANCQDKSDEKNCEVLCLIDQFRCANGQCIGKHKKCDHNVDCSDKSDELDCYPTEEPAPQATNTVGSVIGVIVTIFVSGTVYFICQRMLCPRMKGDGETMTNDYVVHGPASVPLGYVPHPSSLSGSLPGMSRGKSMISSLSIMGGSSGPPYDRAHVTGASSSSSSSTKGTYFPAILNPPPSPATERSHYTMEFGYSSNSPSTHRSYSYRPYSYRHFAPPTTPCSTDVCDSDYAPSRRMTSVATAKGYTSDLNYDSEPVPPPPTPRSQYLSAEENYESCPPSPYTERSYSHHLYPPPPSPCTDSS

SEQ ID NO: 50 - protein, 763 aa, synthetic construct
  REGION 1..763: note = MSLN27 CAR
EVQLVESGGGLVQPGGSLRLSCAASGLIFSTNAMGWFRQAPGKGRELVAAISWRGGYTYYPDSVEGRFTISRDNAKRMVYLQMNSLRAEDTAVYYCAAGTARIDYLSQDGYNYWGQGTQVTVSSTTTPAPRPPTPAPTIASQPLSLRPEACRPAAGGAVHTRGLDFACDIYIWAPLAGTCGVLLLSLVITLYCKRGRKKLLYIFKQPFMRPVQTTQEEDGCSCRFPEEEEGGCELRVKFSRSADAPAYQQGQNQLYNELNLGRREEYDVLDKRRGRDPEMGGKPRRKNPQEGLYNELQKDKMAEAYSEIGMKGERRRGKGHDGLYQGLSTATKDTYDALHMQALPPREGRGSLLTCGDVEENPGPMGAVLRSLLACSFCVLLRAEQKLISEEDLEPPTCSPQQFTCFTGEIDCIPVAWRCDGFTECEDHSDELNCPVCSESQFQCASGQCIDGALRCNGDANCQDKSDEKNCEVLCLIDQFRCANGQCIGKHKKCDHNVDCSDKSDELDCYPTEEPAPQATNTVGSVIGVIVTIFVSGTVYFICQRMLCPRMKGDGETMTNDYVVHGPASVPLGYVPHPSSLSGSLPGMSRGKSMISSLSIMGGSSGPPYDRAHVTGASSSSSSSTKGTYFPAILNPPPSPATERSHYTMEFGYSSNSPSTHRSYSYRPYSYRHFAPPTTPCSTDVCDSDYAPSRRMTSVATAKGYTSDLNYDSEPVPPPPTPRSQYLSAEENYESCPPSPYTERSYSHHLYPPPPSPCTDSS

SEQ ID NO: 51 - protein, 767 aa, synthetic construct
  REGION 1..767: note = MSLN36 CAR
EVQLVESGGGLVQPGGSLRLSCAASGITFSNYVMGWFRQAPGKGRELVAAITASGGNTYYPDSVEGRFTISRDNAKRMVYLQMNSLRAEDTAVYYCAAKRAYWGSDGDYQGYYYYDYWGQGTQVTVSSTTTPAPRPPTPAPTIASQPLSLRPEACRPAAGGAVHTRGLDFACDIYIWAPLAGTCGVLLLSLVITLYCKRGRKKLLYIFKQPFMRPVQTTQEEDGCSCRFPEEEEGGCELRVKFSRSADAPAYQQGQNQLYNELNLGRREEYDVLDKRRGRDPEMGGKPRRKNPQEGLYNELQKDKMAEAYSEIGMKGERRRGKGHDGLYQGLSTATKDTYDALHMQALPPREGRGSLLTCGDVEENPGPMGAVLRSLLACSFCVLLRAEQKLISEEDLEPPTCSPQQFTCFTGEIDCIPVAWRCDGFTECEDHSDELNCPVCSESQFQCASGQCIDGALRCNGDANCQDKSDEKNCEVLCLIDQFRCANGQCIGKHKKCDHNVDCSDKSDELDCYPTEEPAPQATNTVGSVIGVIVTIFVSGTVYFICQRMLCPRMKGDGETMTNDYVVHGPASVPLGYVPHPSSLSGSLPGMSRGKSMISSLSIMGGSSGPPYDRAHVTGASSSSSSSTKGTYFPAILNPPPSPATERSHYTMEFGYSSNSPSTHRSYSYRPYSYRHFAPPTTPCSTDVCDSDYAPSRRMTSVATAKGYTSDLNYDSEPVPPPPTPRSQYLSAEENYESCPPSPYTERSYSHHLYPPPPSPCTDSS

SEQ ID NO: 52 - protein, 767 aa, synthetic construct
  REGION 1..767: note = MSLN41 CAR
EVQLVESGGGLVQPGGSLRLSCAASGRTFSYNAMGWFRQAPGKGRELVAAITWRGGYTYYPDSVEGRFTISRDNAKRMVYLQMNSLRAEDTAVYYCAAATARVYADDSYLNESGYDYWGQGTQVTVSSTTTPAPRPPTPAPTIASQPLSLRPEACRPAAGGAVHTRGLDFACDIYIWAPLAGTCGVLLLSLVITLYCKRGRKKLLYIFKQPFMRPVQTTQEEDGCSCRFPEEEEGGCELRVKFSRSADAPAYQQGQNQLYNELNLGRREEYDVLDKRRGRDPEMGGKPRRKNPQEGLYNELQKDKMAEAYSEIGMKGERRRGKGHDGLYQGLSTATKDTYDALHMQALPPREGRGSLLTCGDVEENPGPMGAVLRSLLACSFCVLLRAEQKLISEEDLEPPTCSPQQFTCFTGEIDCIPVAWRCDGFTECEDHSDELNCPVCSESQFQCASGQCIDGALRCNGDANCQDKSDEKNCEVLCLIDQFRCANGQCIGKHKKCDHNVDCSDKSDELDCYPTEEPAPQATNTVGSVIGVIVTIFVSGTVYFICQRMLCPRMKGDGETMTNDYVVHGPASVPLGYVPHPSSLSGSLPGMSRGKSMISSLSIMGGSSGPPYDRAHVTGASSSSSSSTKGTYFPAILNPPPSPATERSHYTMEFGYSSNSPSTHRSYSYRPYSYRHFAPPTTPCSTDVCDSDYAPSRRMTSVATAKGYTSDLNYDSEPVPPPPTPRSQYLSAEENYESCPPSPYTERSYSHHLYPPPPSPCTDSS

SEQ ID NO: 53 - protein, 767 aa, synthetic construct
  REGION 1..767: note = MSLN42 CAR
EVQLVESGGGLVQPGGSLRLSCAASGRTLSSNVMGWFRQAPGKGRELVAAITPRGSGTYYPDSVEGRFTISRDNAKRMVYLQMNSLRAEDTAVYYCAARFAPDPAFSVYWSENYYDYWGQGTQVTVSSTTTPAPRPPTPAPTIASQPLSLRPEACRPAAGGAVHTRGLDFACDIYIWAPLAGTCGVLLLSLVITLYCKRGRKKLLYIFKQPFMRPVQTTQEEDGCSCRFPEEEEGGCELRVKFSRSADAPAYQQGQNQLYNELNLGRREEYDVLDKRRGRDPEMGGKPRRKNPQEGLYNELQKDKMAEAYSEIGMKGERRRGKGHDGLYQGLSTATKDTYDALHMQALPPREGRGSLLTCGDVEENPGPMGAVLRSLLACSFCVLLRAEQKLISEEDLEPPTCSPQQFTCFTGEIDCIPVAWRCDGFTECEDHSDELNCPVCSESQFQCASGQCIDGALRCNGDANCQDKSDEKNCEVLCLIDQFRCANGQCIGKHKKCDHNVDCSDKSDELDCYPTEEPAPQATNTVGSVIGVIVTIFVSGTVYFICQRMLCPRMKGDGETMTNDYVVHGPASVPLGYVPHPSSLSGSLPGMSRGKSMISSLSIMGGSSGPPYDRAHVTGASSSSSSSTKGTYFPAILNPPPSPATERSHYTMEFGYSSNSPSTHRSYSYRPYSYRHFAPPTTPCSTDVCDSDYAPSRRMTSVATAKGYTSDLNYDSEPVPPPPTPRSQYLSAEENYESCPPSPYTERSYSHHLYPPPPSPCTDSS

SEQ ID NO: 54 - protein, 232 aa, synthetic construct
  REGION 1..232: note = Fc region
EPKSCDKTHTCPPCPAPELLGGPSVFLFPPKPKDTLMISRTPEVTCVVVDVSHEDPEVKFNWYVDGVEVHNAKTKPREEQYNSTYRVVSVLTVLHQDWLNGKEYKCKVSNKALPAPIEKTISKAKGQPREPQVYTLPPSRDELTKNQVSLTCLVKGFYPSDIAVEWESNGQPENNYKTTPPVLDSDGSFFLYSKLTVDKSRWQQGNVFSCSVMHEALHNHYTQKSLSLSPGK

SEQ ID NO: 55 - protein, 11 aa, synthetic construct
  REGION 1..11: note = P4 HCDR3
GMMTYYYGMDV

SEQ ID NO: 56 - protein, 18 aa, synthetic construct
  REGION 1..18: note = P4 HCDR2
RTYYRSKWYNDYAVSVKS

SEQ ID NO: 57 - protein, 7 aa, synthetic construct
  REGION 1..7: note = P4 HCDR1
SNSATWN

SEQ ID NO: 58 - protein, 123 aa, synthetic construct
  REGION 1..123: note = P4 VH
QVQLQQSGPGLVTPSQTLSLTCAISGDSVSSNSATWNWIRQSPSRGLEWLGRTYYRSKWYNDYAVSVKSRMSINPDTSKNQFSLQLNSVTPEDTAVYYCARGMMTYYYGMDVWGQGTTVTVSS

SEQ ID NO: 59 - protein, 9 aa, synthetic construct
  REGION 1..9: note = P4 LCDR3
MIWHSSAAV

SEQ ID NO: 60 - protein, 11 aa, synthetic construct
  REGION 1..11: note = P4 LCDR2
YKSDSDKQQGS

SEQ ID NO: 61 - protein, 14 aa, synthetic construct
  REGION 1..14: note = P4 LCDR1
TLRSGINVGPYRIY

SEQ ID NO: 62 - protein, 116 aa, synthetic construct
  REGION 1..116: note = P4 VL
QPVLTQSSSLSASPGASASLTCTLRSGINVGPYRIYWYQQKPGSPPQYLLNYKSDSDKQQGSGVPSRFSGSKDASANAGVLLISGLRSEDEADYYCMIWHSSAAVFGGGTQLTVLS

SEQ ID NO: 63 - protein, 259 aa, synthetic construct
  REGION 1..259: note = P4 scFv
QVQLQQSGPGLVTPSQTLSLTCAISGDSVSSNSATWNWIRQSPSRGLEWLGRTYYRSKWYNDYAVSVKSRMSINPDTSKNQFSLQLNSVTPEDTAVYYCARGMMTYYYGMDVWGQGTTVTVSSGILGSGGGGSGGGGSGGGGSQPVLTQSSSLSASPGASASLTCTLRSGINVGPYRIYWYQQKPGSPPQYLLNYKSDSDKQQGSGVPSRFSGSKDASANAGVLLISGLRSEDEADYYCMIWHSSAAVFGGGTQLTVLS

SEQ ID NO: 64 - protein, 898 aa, synthetic construct
  REGION 1..898: note = P4 CAR
QVQLQQSGPGLVTPSQTLSLTCAISGDSVSSNSATWNWIRQSPSRGLEWLGRTYYRSKWYNDYAVSVKSRMSINPDTSKNQFSLQLNSVTPEDTAVYYCARGMMTYYYGMDVWGQGTTVTVSSGILGSGGGGSGGGGSGGGGSQPVLTQSSSLSASPGASASLTCTLRSGINVGPYRIYWYQQKPGSPPQYLLNYKSDSDKQQGSGVPSRFSGSKDASANAGVLLISGLRSEDEADYYCMIWHSSAAVFGGGTQLTVLSTTTPAPRPPTPAPTIASQPLSLRPEACRPAAGGAVHTRGLDFACDIYIWAPLAGTCGVLLLSLVITLYCKRGRKKLLYIFKQPFMRPVQTTQEEDGCSCRFPEEEEGGCELRVKFSRSADAPAYQQGQNQLYNELNLGRREEYDVLDKRRGRDPEMGGKPRRKNPQEGLYNELQKDKMAEAYSEIGMKGERRRGKGHDGLYQGLSTATKDTYDALHMQALPPREGRGSLLTCGDVEENPGPMGAVLRSLLACSFCVLLRAEQKLISEEDLEPPTCSPQQFTCFTGEIDCIPVAWRCDGFTECEDHSDELNCPVCSESQFQCASGQCIDGALRCNGDANCQDKSDEKNCEVLCLIDQFRCANGQCIGKHKKCDHNVDCSDKSDELDCYPTEEPAPQATNTVGSVIGVIVTIFVSGTVYFICQRMLCPRMKGDGETMTNDYVVHGPASVPLGYVPHPSSLSGSLPGMSRGKSMISSLSIMGGSSGPPYDRAHVTGASSSSSSSTKGTYFPAILNPPPSPATERSHYTMEFGYSSNSPSTHRSYSYRPYSYRHFAPPTTPCSTDVCDSDYAPSRRMTSVATAKGYTSDLNYDSEPVPPPPTPRSQYLSAEENYESCPPSPYTERSYSHHLYPPPPSPCTDSS

SEQ ID NO: 65 - protein, 15 aa, synthetic construct
  REGION 1..15: note = MSLN10 HCDR3; MSLN27 HCDR3
  SITE 1: note = misc_feature - Xaa = Gly or Arg
  SITE 2: note = misc_feature - Xaa = Arg or Thr
  SITE 3: note = misc_feature - Xaa = Ala or Ile
  SITE 4: note = misc_feature - Xaa = Gly or Arg
  SITE 5: note = misc_feature - Xaa = Ile or Pro
  SITE 6: note = misc_feature - Xaa = Asp or Val
  SITE 8: note = misc_feature - Xaa = Asp or Leu
  SITE 9: note = misc_feature - Xaa = Pro or Ser
  SITE 10: note = misc_feature - Xaa = Gln or Tyr
  SITE 11: note = misc_feature - Xaa = Asp or Ser
  SITE 12: note = misc_feature - Xaa = Gly or Val
XXXXXXYXXXXXYNY

SEQ ID NO: 66 - protein, 19 aa, synthetic construct
  REGION 1..19: note = MSLN36 HCDR3; MSLN41 HCDR3; MSLN42 HCDR3
  SITE 1: note = misc_feature - Xaa = Ala, Lys or Arg
  SITE 2: note = misc_feature - Xaa = Phe, Arg or Thr
  SITE 4: note = misc_feature - Xaa = Pro, Arg or Tyr
  SITE 5: note = misc_feature - Xaa = Asp, Val or Trp
  SITE 6: note = misc_feature - Xaa = Gly, Pro or Tyr
  SITE 7: note = misc_feature - Xaa = Ala or Ser
  SITE 8: note = misc_feature - Xaa = Asp or Phe
  SITE 9: note = misc_feature - Xaa = Asp, Gly or Ser
  SITE 10: note = misc_feature - Xaa = Asp, Ser or Val
  SITE 12: note = misc_feature - Xaa = Leu, Gln or Trp
  SITE 13: note = misc_feature - Xaa = Gly, Asn or Ser
  SITE 14: note = misc_feature - Xaa = Glu or Tyr
  SITE 15: note = misc_feature - Xaa = Asn, Ser or Tyr
  SITE 16: note = misc_feature - Xaa = Gly or Tyr
XXAXXXXXXXYXXXXXYDY

SEQ ID NO: 67 - protein, 17 aa, synthetic construct
  REGION 1..17: note = MSLN16 HCDR2; MSLN3 HCDR2; MSLN10 HCDR2; MSLN27 HCDR2; MSLN36 HCDR2; MSLN41 HCDR2; MSLN42 HCDR2
  SITE 1: note = misc_feature - Xaa = Ala, Gly or Tyr
  SITE 3: note = misc_feature - Xaa = Ser or Thr
  SITE 4: note = misc_feature - Xaa = Ala, Pro, Ser or Trp
  SITE 5: note = misc_feature - Xaa = Gly, Arg or Ser
  SITE 7: note = misc_feature - Xaa = Gly or Ser
  SITE 8: note = misc_feature - Xaa = Gly, Asn, Arg, Ser or Tyr
XIXXXGXXTYYPDSVEG

SEQ ID NO: 68 - skipped

SEQ ID NO: 69 - protein, 124 aa, synthetic construct
  REGION 1..124: note = MSLN10 VHH; MSLN27 VHH
  SITE 27: note = misc_feature - Xaa = Asp or Leu
  SITE 28: note = misc_feature - Xaa = Ile or Thr
  SITE 29: note = misc_feature - Xaa = Phe or Leu
  SITE 32: note = misc_feature - Xaa = Asn or Tyr
  SITE 50: note = misc_feature - Xaa = Ala or Gly
  SITE 52: note = misc_feature - Xaa = Ser or Thr
  SITE 53: note = misc_feature - Xaa = Ser or Trp
  SITE 54: note = misc_feature - Xaa = Arg or Ser
  SITE 56: note = misc_feature - Xaa = Gly or Ser
  SITE 57: note = misc_feature - Xaa = Gly or Tyr
  SITE 99: note = misc_feature - Xaa = Gly or Arg
  SITE 100: note = misc_feature - Xaa = Arg or Thr
  SITE 101: note = misc_feature - Xaa = Ala or Ile
  SITE 102: note = misc_feature - Xaa = Gly or Arg
  SITE 103: note = misc_feature - Xaa = Ile or Pro
  SITE 104: note = misc_feature - Xaa = Asp or Val
  SITE 106: note = misc_feature - Xaa = Asp or Leu
  SITE 107: note = misc_feature - Xaa = Pro or Ser
  SITE 108: note = misc_feature - Xaa = Gln or Tyr
  SITE 109: note = misc_feature - Xaa = Asp or Ser
  SITE 110: note = misc_feature - Xaa = Gly or Val
EVQLVESGGGLVQPGGSLRLSCAASGXXXSTXAMGWFRQAPGKGRELVAXIXXXGXXTYYPDSVEGRFTISRDNAKRMVYLQMNSLRAEDTAVYYCAAXXXXXXYXXXXXYNYWGQGTQVTVSS

SEQ ID NO: 70 - protein, 128 aa, synthetic construct
  REGION 1..128: note = MSLN36 VHH; MSLN41 VHH; MSLN42 VHH
  SITE 27: note = misc_feature - Xaa = Ile or Arg
  SITE 29: note = misc_feature - Xaa = Phe or Leu
  SITE 31: note = misc_feature - Xaa = Asn, Ser or Tyr
  SITE 32: note = misc_feature - Xaa = Asn or Tyr
  SITE 33: note = misc_feature - Xaa = Ala or Val
  SITE 53: note = misc_feature - Xaa = Ala, Pro or Trp
  SITE 54: note = misc_feature - Xaa = Arg or Ser
  SITE 56: note = misc_feature - Xaa = Gly or Ser
  SITE 57: note = misc_feature - Xaa = Gly, Asn or Tyr
  SITE 99: note = misc_feature - Xaa = Ala, Lys or Arg
  SITE 100: note = misc_feature - Xaa = Phe, Arg or Thr
  SITE 102: note = misc_feature - Xaa = Pro, Arg or Tyr
  SITE 103: note = misc_feature - Xaa = Asp, Val or Trp
  SITE 104: note = misc_feature - Xaa = Gly, Pro or Tyr
  SITE 105: note = misc_feature - Xaa = Ala or Ser
  SITE 106: note = misc_feature - Xaa = Asp or Phe
  SITE 107: note = misc_feature - Xaa = Asp, Gly or Ser
  SITE 108: note = misc_feature - Xaa = Asp, Ser or Val
  SITE 110: note = misc_feature - Xaa = Leu, Gln or Trp
  SITE 111: note = misc_feature - Xaa = Gly, Asn or Ser
  SITE 112: note = misc_feature - Xaa = Glu or Tyr
  SITE 113: note = misc_feature - Xaa = Asn, Ser or Tyr
  SITE 114: note = misc_feature - Xaa = Gly or Tyr
EVQLVESGGGLVQPGGSLRLSCAASGXTXSXXXMGWFRQAPGKGRELVAAITXXGXXTYYPDSVEGRFTISRDNAKRMVYLQMNSLRAEDTAVYYCAAXXAXXXXXXXYXXXXXYDYWGQGTQVTVSS